European Patent Application EP 4 495 115 A1, published January 22, 2025. Title: Tetracyclic compound and use thereof. Applicant: SHANGHAI SHIJIANG BIOTECHNOLOGY CO., LTD. Application EP. The sequence listing filed with the application follows.

SEQUENCE LISTING (3 sequences)

SEQ ID NO: 1 - DNA, 2500 bp, synthetic construct
  source 1..2500: mol_type = other DNA
tatccaagagctatcagcactcccatgtttattgtagcactgttcacaatagccaagatttggaagtactctaagtgtccattagcagatgaatggataaagacaatgtggtaatacacataatggagtactattcagtcataaagaagaattagatcctgtcatttgcaataacatggatggaactggaggtcataatgttgagtgaaataaaccaggcacagaaagacaaactttgcatgttctcacttatttatgggagctaaaaactaaaataactgaactcacagagatagagagtagaaggatggttacgagaggatgggaagggtagcgaggtgggtaggggggatgtggggatcattaatgggtataaaaaatagttagaggccaggcgcagtggctcacgcctgtaatcccagcactttgggaggccgaggtaggcggaacacctgaggagttcaagaccagcctggccaatatgatgaaaccccgtctctactaaaaatacaaaaattagctgggcgtgatggtgtgcacctgtagtcccagctgcttgggaggctgaggcaggagaatcgctggaacccaagaggtgaaggttgcagtgagctgagatcgcgtcactgcactccagcctgggtgacagagtgagactccacatcaaaaaaaaaaaaaaaaagttagaaagattgaataagacctaatatttgctagcacaacagggtgaatatagtaaaaaataatttatttgtaccttcaaaaataactagacaagtataattgggttgtttgtaacacacaaaaaataagtacttgaagtggtggataccccatttaccctgatgtgattattttgtattgcaggcctctatcagaatatctcatgtaacccataaatatatacacctactctgtacccacaaaaagtttttaaaaagaaaaataaatagcaaccgaaaaaaaaagagagggagaaaagaaaaaagaaaaaaaaatcaagtgcctggctgggtagaataaattctaaggccacaatgttactgaccatgggttttttggctctcagtgtatagaaattgacacaaggccaatagtcttcccaaacatgctttactggaacttacgccctggcataagggccacaacaaaagagagagcgaattctctggcttgctgactccttggaaaaaaccggtagggatttttttattaggcaaagcacaggaattgacgtcagaggcaggatgtgctgctgggcaaagcatacgagaagtggggtatgcaggtcagcattacttggttgcaatggttatcttgaggaatgggccaactggtggtctggccagtggcaacaaggctgtaaatcaattattcagcattccttcccaaggtgggacacccggcaacattgtttatctcctaaggccagttcctggaattaagtgaaaggatgactaatggacatgttgtcagtgaggtagtggtgtgggttttgtgaccagtgggaatgcacgaaagaatgctttagcggggagtgagctgaagccaagccccatccctactctgtctcaaagtgagttcagaaaaggggatttaaagaattctttttttttttttttttttttttgagacagagtcttgctctgtcgcccaggctggagtgcagtggcgccatcttggctcactgcaagctccgccccccgggttcatgccattctcctgcctcagcctcccaagtagctgggactgcaggtgcctaccaccaagcccagctaattttttgtattttttttttagtagagacggggtttcaccatgttagccaggatggtctcgatctcctgacctcgtgatctgcccgccttagcctcccaaagtgctgggattacaggcatgagcctccgcccccggccttaaataattcttaaaggaagtaaagttaactttgaaagaactatcaggatttggattgactgaaaggagtggggaagcttagggaggaggtgcttgccagacactgggtcatggcagtggtcggtgaagctgcagttgcctagggcagggatggagagagagtctgggcatgaggagagggtctcgggatgtttggctggactagattttacagaaagccttatccaggcttttaaaattactctttccagacttcatctgagactccttcttcagccaacattccttagccctgaatacatttcctatcctcatctttcccttcttttttttcctttcttttacatgtttaaatttaaaccattcttcgtgaccccttttcttgggagattcatggcaagaacgagaagaatgatggtgcttgttaggggatgtcctgtctctctgaactttggggtcctatgcattaaataattttcctgacgagctcaagtgctccctctggtctacaatccctggcggctggccttcatcccttgggcaagcattgcatacagctcatggccctccctctaccataccc

SEQ ID NO: 2 - DNA, 21 bp, synthetic construct
  source 1..21: mol_type = other DNA
gttcttcatctgcaccataaa

SEQ ID NO: 3 - DNA, 64 bp, synthetic construct
  source 1..64: mol_type = other DNA
gatccgggatgagtccatcaaggaagattcaagagatcttccttgatggactcatccttttttg